European Patent Specification EP 3 571 582 B1, published February 11, 2026. Title: SYSTEMS AND METHODS FOR SUPPORTING MULTIPLE AUTOMATED WORKFLOWS. Applicant: Lifefoundry, Inc. Chao, Rao Zhao, Huimin. The sequence listing filed with the application follows.

SEQUENCE LISTING (1 sequence)

SEQ ID NO: 1 - DNA, 72 bp, Artificial Sequence
  cleaver
ggcagcggagctactaacttcagcctgctgaagcaggctggagatgtggaggagaaccctggacctggcatg